European Patent Application EP 4 159 752 A1, published April 5, 2023. Title: Chimeric Antigen Receptors. Applicant: MolMed S.p.A. The sequence listing filed with the application follows.

SEQUENCE LISTING (40 sequences)

SEQ ID NO: 1 - protein, 222 aa, synthetic construct
  REGION 1..222: note = Spacer LNGFR wild-type long (NWL)
KEACPTGLYTHSGECCKACNLGEGVAQPCGANQTVCEPCLDSVTFSDVVSATEPCKPCTECVGLQSMSAPCVEADDAVCRCAYGYYQDETTGRCEACRVCEAGSGLVFSCQDKQNTVCEECPDGTYSDEANHVDPCLPCTVCEDTERQLRECTRWADAECEEIPGRWITRSTPPEGSDSTAPSTQEPEAPPEQDLIASTVAGVVTTVMGSSQPVVTRGTTDN

SEQ ID NO: 2 - DNA, 666 bp, synthetic construct
  misc_feature 1..666: note = Spacer LNGFR wild-type long (NWL)
  source 1..666: mol_type = other DNA
aaagaggcctgccccaccggcctgtacacccacagcggagagtgctgcaaggcctgcaacctgggagagggcgtggcccagccttgcggcgccaatcagaccgtgtgcgagccctgcctggacagcgtgaccttcagcgacgtggtgtccgccaccgagccctgcaagccttgcaccgagtgtgtgggcctgcagagcatgagcgccccctgcgtggaagccgacgacgccgtgtgtagatgcgcctacggctactaccaggacgagacaaccggcagatgcgaggcctgtagagtgtgcgaggccggcagcggcctggtgttcagttgtcaagacaagcagaataccgtgtgtgaagagtgccccgacggcacctacagcgacgaggccaaccacgtggacccctgcctgccctgcactgtgtgcgaggacaccgagcggcagctgcgcgagtgcacaagatgggccgacgccgagtgcgaagagatccccggcagatggatcaccagaagcaccccccctgagggcagcgacagcaccgcccctagcacccaggaacctgaggcccctcccgagcaggacctgatcgcctctacagtggccggcgtggtgacaaccgtgatgggcagctctcagcccgtggtgacacggggcaccaccgacaat

SEQ ID NO: 3 - protein, 162 aa, synthetic construct
  REGION 1..162: note = Spacer LNGFR wild-type short (NWS)
KEACPTGLYTHSGECCKACNLGEGVAQPCGANQTVCEPCLDSVTFSDVVSATEPCKPCTECVGLQSMSAPCVEADDAVCRCAYGYYQDETTGRCEACRVCEAGSGLVFSCQDKQNTVCEECPDGTYSDEANHVDPCLPCTVCEDTERQLRECTRWADAECEE

SEQ ID NO: 4 - DNA, 486 bp, synthetic construct
  misc_feature 1..486: note = Spacer LNGFR wild-type short (NWS)
  source 1..486: mol_type = other DNA
aaagaggcctgccccaccggcctgtacacccacagcggagagtgctgcaaggcctgcaacctgggagagggcgtggcccagccttgcggcgccaatcagaccgtgtgcgagccctgcctggacagcgtgaccttcagcgacgtggtgtccgccaccgagccctgcaagccttgcaccgagtgtgtgggcctgcagagcatgagcgccccctgcgtggaagccgacgacgccgtgtgtagatgcgcctacggctactaccaggacgagacaaccggcagatgcgaggcctgtagagtgtgcgaggccggcagcggcctggtgttcagttgtcaggacaagcagaacaccgtgtgtgaagagtgccccgacggcacctacagcgacgaggccaaccacgtggacccctgcctgccctgcactgtgtgcgaggacaccgagcggcagctgcgcgagtgcacaagatgggccgacgccgagtgcgaggaa

SEQ ID NO: 5 - protein, 200 aa, synthetic construct
  REGION 1..200: note = Spacer LNGFR mutated long (NML)
KEACPTGLYTHSGECCKACNLGEGVAQPCGANQTVCEPCLDSVTFSDVVSATEPCKPCTECVGLQSMSAPCVEADDAVCRCAYGYYQDETTGRCEACRVCEAGSGLVFSCQDKQNTVCEECPDGTYSDEAARAADAECEEIPGRWITRSTPPEGSDSTAPSTQEPEAPPEQDLIASTVAGVVTTVMGSSQPVVTRGTTDN

SEQ ID NO: 6 - DNA, 600 bp, synthetic construct
  misc_feature 1..600: note = Spacer LNGFR mutated long (NML)
  source 1..600: mol_type = other DNA
aaagaggcctgccccaccggcctgtacacccacagcggagagtgctgcaaggcctgcaacctgggagagggcgtggcccagccttgcggcgccaatcagaccgtgtgcgagccctgcctggacagcgtgaccttcagcgacgtggtgtccgccaccgagccctgcaagccttgcaccgagtgtgtgggcctgcagagcatgagcgccccctgcgtggaagccgacgacgccgtgtgtagatgcgcctacggctactaccaggacgagacaaccggcagatgcgaggcctgtagagtgtgcgaggccggcagcggcctggtgttcagttgtcaagacaagcagaataccgtgtgtgaagagtgccccgacggcacctacagcgacgaagccgccagagccgccgacgccgagtgcgaagagatccccggcagatggatcaccagaagcaccccccctgagggcagcgacagcaccgcccctagcacccaggaacctgaggcccctcccgagcaggacctgatcgcctctacagtggccggcgtggtgacaaccgtgatgggcagctctcagcccgtggtgacacggggcaccaccgacaat

SEQ ID NO: 7 - protein, 140 aa, synthetic construct
  REGION 1..140: note = Spacer LNGFR mutated short (NMS)
KEACPTGLYTHSGECCKACNLGEGVAQPCGANQTVCEPCLDSVTFSDVVSATEPCKPCTECVGLQSMSAPCVEADDAVCRCAYGYYQDETTGRCEACRVCEAGSGLVFSCQDKQNTVCEECPDGTYSDEAARAADAECEE

SEQ ID NO: 8 - DNA, 420 bp, synthetic construct
  misc_feature 1..420: note = Spacer LNGFR mutated short (NMS)
  source 1..420: mol_type = other DNA
aaagaggcctgccccaccggcctgtacacccacagcggagagtgctgcaaggcctgcaacctgggagagggcgtggcccagccttgcggcgccaatcagaccgtgtgcgagccctgcctggacagcgtgaccttcagcgacgtggtgtccgccaccgagccctgcaagccttgcaccgagtgtgtgggcctgcagagcatgagcgccccctgcgtggaagccgacgacgccgtgtgtagatgcgcctacggctactaccaggacgagacaaccggcagatgcgaggcctgtagagtgtgcgaggccggcagcggcctggtgttcagttgtcaggacaagcagaacaccgtgtgtgaagagtgccccgacggcacctacagcgacgaggccgcccgggccgccgacgccgagtgcgaggaa

SEQ ID NO: 9 - protein, 34 aa, Homo sapiens
ACPTGLYTHSGECCKACNLGEGVAQPCGANQTVC

SEQ ID NO: 10 - protein, 42 aa, Homo sapiens
PCLDSVTFSDVVSATEPCKPCTECVGLQSMSAPCVEADDAVC

SEQ ID NO: 11 - protein, 39 aa, Homo sapiens
RCAYGYYQDETTGRCEACRVCEAGSGLVFSCQDKQNTVC

SEQ ID NO: 12 - protein, 41 aa, Homo sapiens
ECPDGTYSDEANHVDPCLPCTVCEDTERQLRECTRWADAEC

SEQ ID NO: 13 - protein, 25 aa, Homo sapiens
NHVDPCLPCTVCEDTERQLRECTRW

SEQ ID NO: 14 - protein, 427 aa, Homo sapiens
MGAGATGRAMDGPRLLLLLLLGVSLGGAKEACPTGLYTHSGECCKACNLGEGVAQPCGANQTVCEPCLDSVTFSDVVSATEPCKPCTECVGLQSMSAPCVEADDAVCRCAYGYYQDETTGRCEACRVCEAGSGLVFSCQDKQNTVCEECPDGTYSDEANHVDPCLPCTVCEDTERQLRECTRWADAECEEIPGRWITRSTPPEGSDSTAPSTQEPEAPPEQDLIASTVAGVVTTVMGSSQPVVTRGTTDNLIPVYCSILAAVVVGLVAYIAFKRWNSCKQNKQGANSRPVNQTPPPEGEKLHSDSGISVDSQSLHDQQPHTQTASGQALKGDGGLYSSLPPAKREEVEKLLNGSAGDTWRHLAGELGYQPEHIDSFTHEACPVRALLASWATQDSATLDALLAALRRIQRADLVESLCSESTATSPV

SEQ ID NO: 15 - DNA, 2046 bp, synthetic construct
  misc_feature 1..2046: note = CD44v6-specific second-generation CAR construct sequence,CD44v6-CAR.28z
  source 1..2046: mol_type = other DNA
atggaagcccctgcccagctgctgttcctgctgctgctgtggctgcccgacaccaccggcgagatcgtgctgacacagagccccgccaccctgtctctgagccctggcgagagagccaccctgagctgtagcgccagcagcagcatcaactacatctactggctgcagcagaagcccggccaggcccccagaatcctgatctacctgaccagcaacctggccagcggcgtgcccgccagattttctggcagcggcagcggcaccgacttcaccctgaccatcagcagcctggaacccgaggacttcgccgtgtactactgcctgcagtggtccagcaaccccctgaccttcggcggaggcaccaaggtggaaatcaagcggggtggtggtggttctggtggtggtggttctggcggcggcggctccggtggtggtggatctgaggtgcagctggtggaaagcggcggaggcctggtcaagcctggcggcagcctgagactgagctgtgccgccagcggcttcaccttcagcagctacgacatgagctgggtccgacaggctccaggcaagggactggaatgggtgtccaccatcagcagcggcggcagctacacctactacctggacagcatcaagggccggttcaccatcagccgggacaacgccaagaacagcctgtacctgcagatgaacagcctgcgggccgaggacaccgccgtctactactgtgcccggcagggcctcgactactggggcagaggcaccctggtcaccgtgtccagcggggatcccgccgagcccaaatctcctgacaaaactcacacatgcccaccgtgcccagcacctgaactcctggggggaccgtcagtcttcctcttccccccaaaacccaaggacaccctcatgatctcccggacccctgaggtcacatgcgtggtggtggacgtgagccacgaagaccctgaggtcaagttcaactggtacgtggacggcgtggaggtgcataatgccaagacaaagccgcgggaggagcagtacaacagcacgtaccgtgtggtcagcgtcctcaccgtcctgcaccaggactggctgaatggcaaggagtacaagtgcaaggtctccaacaaagccctcccagcccccatcgagaaaaccatctccaaagccaaagggcagccccgagaaccacaggtgtacaccctgcccccatcccgggatgagctgaccaagaaccaggtcagcctgacctgcctggtcaaaggcttctatcccagcgacatcgccgtggagtgggagagcaatgggcaaccggagaacaactacaagaccacgcctcccgtgctggactccgacggctccttcttcctctacagcaagctcaccgtggacaagagcaggtggcagcaggggaacgtcttctcatgctccgtgatgcatgaggctctgcacaaccactacacgcagaagagcctctccctgtctccgggtaaaaaagatcccaaattttgggtgctggtggtggttggtggagtcctggcttgctatagcttgctagtaacagtggcctttattattttctgggtgaggagtaagaggagcaggctcctgcacagtgactacatgaacatgactccccgccgccccgggcccacccgcaagcattaccagccctatgccccaccacgcgacttcgcagcctatcgctccagagtgaagttcagcaggagcgcagacgcccccgcgtaccagcagggccagaaccagctctataacgagctcaatctaggacgaagagaggagtacgatgttttggacaagagacgtggccgggaccctgagatggggggaaagccgagaaggaagaaccctcaggaaggcctgtacaatgaactgcagaaagataagatggcggaggcctacagtgagattgggatgaaaggcgagcgccggaggggcaaggggcacgatggcctttaccagggtctcagtacagccaccaaggacacctacgacgcccttcacatgcaggccctgccccctcgctaa

SEQ ID NO: 16 - protein, 681 aa, synthetic construct
  REGION 1..681: note = CD44v6-CAR.28z protein
MEAPAQLLFLLLLWLPDTTGEIVLTQSPATLSLSPGERATLSCSASSSINYIYWLQQKPGQAPRILIYLTSNLASGVPARFSGSGSGTDFTLTISSLEPEDFAVYYCLQWSSNPLTFGGGTKVEIKRGGGGSGGGGSGGGGSGGGGSEVQLVESGGGLVKPGGSLRLSCAASGFTFSSYDMSWVRQAPGKGLEWVSTISSGGSYTYYLDSIKGRFTISRDNAKNSLYLQMNSLRAEDTAVYYCARQGLDYWGRGTLVTVSSGDPAEPKSPDKTHTCPPCPAPELLGGPSVFLFPPKPKDTLMISRTPEVTCVVVDVSHEDPEVKFNWYVDGVEVHNAKTKPREEQYNSTYRVVSVLTVLHQDWLNGKEYKCKVSNKALPAPIEKTISKAKGQPREPQVYTLPPSRDELTKNQVSLTCLVKGFYPSDIAVEWESNGQPENNYKTTPPVLDSDGSFFLYSKLTVDKSRWQQGNVFSCSVMHEALHNHYTQKSLSLSPGKKDPKFWVLVVVGGVLACYSLLVTVAFIIFWVRSKRSRLLHSDYMNMTPRRPGPTRKHYQPYAPPRDFAAYRSRVKFSRSADAPAYQQGQNQLYNELNLGRREEYDVLDKRRGRDPEMGGKPRRKNPQEGLYNELQKDKMAEAYSEIGMKGERRRGKGHDGLYQGLSTATKDTYDALHMQALPPR

SEQ ID NO: 17 - protein, 261 aa, synthetic construct
  REGION 1..261: note = CD44v6-specific single-chain fragment
MEAPAQLLFLLLLWLPDTTGEIVLTQSPATLSLSPGERATLSCSASSSINYIYWLQQKPGQAPRILIYLTSNLASGVPARFSGSGSGTDFTLTISSLEPEDFAVYYCLQWSSNPLTFGGGTKVEIKRGGGGSGGGGSGGGGSGGGGSEVQLVESGGGLVKPGGSLRLSCAASGFTFSSYDMSWVRQAPGKGLEWVSTISSGGSYTYYLDSIKGRFTISRDNAKNSLYLQMNSLRAEDTAVYYCARQGLDYWGRGTLVTVSS

SEQ ID NO: 18 - protein, 68 aa, Homo sapiens
FWVLVVVGGVLACYSLLVTVAFIIFWVRSKRSRLLHSDYMNMTPRRPGPTRKHYQPYAPPRDFAAYRS

SEQ ID NO: 19 - protein, 222 aa, Homo sapiens; identical to SEQ ID NO: 1

SEQ ID NO: 20 - protein, 113 aa, Homo sapiens
RVKFSRSADAPAYQQGQNQLYNELNLGRREEYDVLDKRRGRDPEMGGKPQRRKNPQEGLYNELQKDKMAEAYSEIGMKGERRRGKGHDGLYQGLSTATKDTYDALHMQALPPR

SEQ ID NO: 21 - protein, 669 aa, synthetic construct
  REGION 1..669: note = CD44v6-CAR28z with spacer LNGFR wild-type long (NWL)
MEAPAQLLFLLLLWLPDTTGEIVLTQSPATLSLSPGERATLSCSASSSINYIYWLQQKPGQAPRILIYLTSNLASGVPARFSGSGSGTDFTLTISSLEPEDFAVYYCLQWSSNPLTFGGGTKVEIKRGGGGSGGGGSGGGGSGGGGSEVQLVESGGGLVKPGGSLRLSCAASGFTFSSYDMSWVRQAPGKGLEWVSTISSGGSYTYYLDSIKGRFTISRDNAKNSLYLQMNSLRAEDTAVYYCARQGLDYWGRGTLVTVSSGDPKEACPTGLYTHSGECCKACNLGEGVAQPCGANQTVCEPCLDSVTFSDVVSATEPCKPCTECVGLQSMSAPCVEADDAVCRCAYGYYQDETTGRCEACRVCEAGSGLVFSCQDKQNTVCEECPDGTYSDEANHVDPCLPCTVCEDTERQLRECTRWADAECEEIPGRWITRSTPPEGSDSTAPSTQEPEAPPEQDLIASTVAGVVTTVMGSSQPVVTRGTTDNPKFWVLVVVGGVLACYSLLVTVAFIIFWVRSKRSRLLHSDYMNMTPRRPGPTRKHYQPYAPPRDFAAYRSRVKFSRSADAPAYQQGQNQLYNELNLGRREEYDVLDKRRGRDPEMGGKPQRRKNPQEGLYNELQKDKMAEAYSEIGMKGERRRGKGHDGLYQGLSTATKDTYDALHMQALPPR

SEQ ID NO: 22 - protein, 609 aa, synthetic construct
  REGION 1..609: note = CD44v6-CAR28z with spacer LNGFR wild-type short (NWS)
MEAPAQLLFLLLLWLPDTTGEIVLTQSPATLSLSPGERATLSCSASSSINYIYWLQQKPGQAPRILIYLTSNLASGVPARFSGSGSGTDFTLTISSLEPEDFAVYYCLQWSSNPLTFGGGTKVEIKRGGGGSGGGGSGGGGSGGGGSEVQLVESGGGLVKPGGSLRLSCAASGFTFSSYDMSWVRQAPGKGLEWVSTISSGGSYTYYLDSIKGRFTISRDNAKNSLYLQMNSLRAEDTAVYYCARQGLDYWGRGTLVTVSSGDPKEACPTGLYTHSGECCKACNLGEGVAQPCGANQTVCEPCLDSVTFSDVVSATEPCKPCTECVGLQSMSAPCVEADDAVCRCAYGYYQDETTGRCEACRVCEAGSGLVFSCQDKQNTVCEECPDGTYSDEANHVDPCLPCTVCEDTERQLRECTRWADAECEEPKFWVLVVVGGVLACYSLLVTVAFIIFWVRSKRSRLLHSDYMNMTPRRPGPTRKHYQPYAPPRDFAAYRSRVKFSRSADAPAYQQGQNQLYNELNLGRREEYDVLDKRRGRDPEMGGKPQRRKNPQEGLYNELQKDKMAEAYSEIGMKGERRRGKGHDGLYQGLSTATKDTYDALHMQALPPR

SEQ ID NO: 23 - protein, 647 aa, synthetic construct
  REGION 1..647: note = CD44v6-CAR28z with spacer LNGFR mutated long (NML)
MEAPAQLLFLLLLWLPDTTGEIVLTQSPATLSLSPGERATLSCSASSSINYIYWLQQKPGQAPRILIYLTSNLASGVPARFSGSGSGTDFTLTISSLEPEDFAVYYCLQWSSNPLTFGGGTKVEIKRGGGGSGGGGSGGGGSGGGGSEVQLVESGGGLVKPGGSLRLSCAASGFTFSSYDMSWVRQAPGKGLEWVSTISSGGSYTYYLDSIKGRFTISRDNAKNSLYLQMNSLRAEDTAVYYCARQGLDYWGRGTLVTVSSGDPKEACPTGLYTHSGECCKACNLGEGVAQPCGANQTVCEPCLDSVTFSDVVSATEPCKPCTECVGLQSMSAPCVEADDAVCRCAYGYYQDETTGRCEACRVCEAGSGLVFSCQDKQNTVCEECPDGTYSDEAARAADAECEEIPGRWITRSTPPEGSDSTAPSTQEPEAPPEQDLIASTVAGVVTTVMGSSQPVVTRGTTDNPKFWVLVVVGGVLACYSLLVTVAFIIFWVRSKRSRLLHSDYMNMTPRRPGPTRKHYQPYAPPRDFAAYRSRVKFSRSADAPAYQQGQNQLYNELNLGRREEYDVLDKRRGRDPEMGGKPQRRKNPQEGLYNELQKDKMAEAYSEIGMKGERRRGKGHDGLYQGLSTATKDTYDALHMQALPPR

SEQ ID NO: 24 - protein, 587 aa, synthetic construct
  REGION 1..587: note = CD44v6-CAR28z with spacer LNGFR mutated short (NMS)
MEAPAQLLFLLLLWLPDTTGEIVLTQSPATLSLSPGERATLSCSASSSINYIYWLQQKPGQAPRILIYLTSNLASGVPARFSGSGSGTDFTLTISSLEPEDFAVYYCLQWSSNPLTFGGGTKVEIKRGGGGSGGGGSGGGGSGGGGSEVQLVESGGGLVKPGGSLRLSCAASGFTFSSYDMSWVRQAPGKGLEWVSTISSGGSYTYYLDSIKGRFTISRDNAKNSLYLQMNSLRAEDTAVYYCARQGLDYWGRGTLVTVSSGDPKEACPTGLYTHSGECCKACNLGEGVAQPCGANQTVCEPCLDSVTFSDVVSATEPCKPCTECVGLQSMSAPCVEADDAVCRCAYGYYQDETTGRCEACRVCEAGSGLVFSCQDKQNTVCEECPDGTYSDEAARAADAECEEPKFWVLVVVGGVLACYSLLVTVAFIIFWVRSKRSRLLHSDYMNMTPRRPGPTRKHYQPYAPPRDFAAYRSRVKFSRSADAPAYQQGQNQLYNELNLGRREEYDVLDKRRGRDPEMGGKPQRRKNPQEGLYNELQKDKMAEAYSEIGMKGERRRGKGHDGLYQGLSTATKDTYDALHMQALPPR

SEQ ID NO: 25 - protein, 668 aa, synthetic construct
  REGION 1..668: note = CD44v6-CAR28z with spacer LNGFR wild-type long (NWL)
MEAPAQLLFLLLLWLPDTTGEIVLTQSPATLSLSPGERATLSCSASSSINYIYWLQQKPGQAPRILIYLTSNLASGVPARFSGSGSGTDFTLTISSLEPEDFAVYYCLQWSSNPLTFGGGTKVEIKRGGGGSGGGGSGGGGSGGGGSEVQLVESGGGLVKPGGSLRLSCAASGFTFSSYDMSWVRQAPGKGLEWVSTISSGGSYTYYLDSIKGRFTISRDNAKNSLYLQMNSLRAEDTAVYYCARQGLDYWGRGTLVTVSSGDPKEACPTGLYTHSGECCKACNLGEGVAQPCGANQTVCEPCLDSVTFSDVVSATEPCKPCTECVGLQSMSAPCVEADDAVCRCAYGYYQDETTGRCEACRVCEAGSGLVFSCQDKQNTVCEECPDGTYSDEANHVDPCLPCTVCEDTERQLRECTRWADAECEEIPGRWITRSTPPEGSDSTAPSTQEPEAPPEQDLIASTVAGVVTTVMGSSQPVVTRGTTDNPKFWVLVVVGGVLACYSLLVTVAFIIFWVRSKRSRLLHSDYMNMTPRRPGPTRKHYQPYAPPRDFAAYRSRVKFSRSADAPAYQQGQNQLYNELNLGRREEYDVLDKRRGRDPEMGGKPRRKNPQEGLYNELQKDKMAEAYSEIGMKGERRRGKGHDGLYQGLSTATKDTYDALHMQALPPR

SEQ ID NO: 26 - protein, 608 aa, synthetic construct
  REGION 1..608: note = CD44v6-CAR28z with spacer LNGFR wild-type short (NWS)
MEAPAQLLFLLLLWLPDTTGEIVLTQSPATLSLSPGERATLSCSASSSINYIYWLQQKPGQAPRILIYLTSNLASGVPARFSGSGSGTDFTLTISSLEPEDFAVYYCLQWSSNPLTFGGGTKVEIKRGGGGSGGGGSGGGGSGGGGSEVQLVESGGGLVKPGGSLRLSCAASGFTFSSYDMSWVRQAPGKGLEWVSTISSGGSYTYYLDSIKGRFTISRDNAKNSLYLQMNSLRAEDTAVYYCARQGLDYWGRGTLVTVSSGDPKEACPTGLYTHSGECCKACNLGEGVAQPCGANQTVCEPCLDSVTFSDVVSATEPCKPCTECVGLQSMSAPCVEADDAVCRCAYGYYQDETTGRCEACRVCEAGSGLVFSCQDKQNTVCEECPDGTYSDEANHVDPCLPCTVCEDTERQLRECTRWADAECEEPKFWVLVVVGGVLACYSLLVTVAFIIFWVRSKRSRLLHSDYMNMTPRRPGPTRKHYQPYAPPRDFAAYRSRVKFSRSADAPAYQQGQNQLYNELNLGRREEYDVLDKRRGRDPEMGGKPRRKNPQEGLYNELQKDKMAEAYSEIGMKGERRRGKGHDGLYQGLSTATKDTYDALHMQALPPR

SEQ ID NO: 27 - protein, 646 aa, synthetic construct
  REGION 1..646: note = CD44v6-CAR28z with spacer LNGFR mutated long (NWL)
MEAPAQLLFLLLLWLPDTTGEIVLTQSPATLSLSPGERATLSCSASSSINYIYWLQQKPGQAPRILIYLTSNLASGVPARFSGSGSGTDFTLTISSLEPEDFAVYYCLQWSSNPLTFGGGTKVEIKRGGGGSGGGGSGGGGSGGGGSEVQLVESGGGLVKPGGSLRLSCAASGFTFSSYDMSWVRQAPGKGLEWVSTISSGGSYTYYLDSIKGRFTISRDNAKNSLYLQMNSLRAEDTAVYYCARQGLDYWGRGTLVTVSSGDPKEACPTGLYTHSGECCKACNLGEGVAQPCGANQTVCEPCLDSVTFSDVVSATEPCKPCTECVGLQSMSAPCVEADDAVCRCAYGYYQDETTGRCEACRVCEAGSGLVFSCQDKQNTVCEECPDGTYSDEAARAADAECEEIPGRWITRSTPPEGSDSTAPSTQEPEAPPEQDLIASTVAGVVTTVMGSSQPVVTRGTTDNPKFWVLVVVGGVLACYSLLVTVAFIIFWVRSKRSRLLHSDYMNMTPRRPGPTRKHYQPYAPPRDFAAYRSRVKFSRSADAPAYQQGQNQLYNELNLGRREEYDVLDKRRGRDPEMGGKPRRKNPQEGLYNELQKDKMAEAYSEIGMKGERRRGKGHDGLYQGLSTATKDTYDALHMQALPPR

SEQ ID NO: 28 - protein, 586 aa, synthetic construct
  REGION 1..586: note = CD44v6-CAR28z with spacer LNGFR mutated short (NWL)
MEAPAQLLFLLLLWLPDTTGEIVLTQSPATLSLSPGERATLSCSASSSINYIYWLQQKPGQAPRILIYLTSNLASGVPARFSGSGSGTDFTLTISSLEPEDFAVYYCLQWSSNPLTFGGGTKVEIKRGGGGSGGGGSGGGGSGGGGSEVQLVESGGGLVKPGGSLRLSCAASGFTFSSYDMSWVRQAPGKGLEWVSTISSGGSYTYYLDSIKGRFTISRDNAKNSLYLQMNSLRAEDTAVYYCARQGLDYWGRGTLVTVSSGDPKEACPTGLYTHSGECCKACNLGEGVAQPCGANQTVCEPCLDSVTFSDVVSATEPCKPCTECVGLQSMSAPCVEADDAVCRCAYGYYQDETTGRCEACRVCEAGSGLVFSCQDKQNTVCEECPDGTYSDEAARAADAECEEPKFWVLVVVGGVLACYSLLVTVAFIIFWVRSKRSRLLHSDYMNMTPRRPGPTRKHYQPYAPPRDFAAYRSRVKFSRSADAPAYQQGQNQLYNELNLGRREEYDVLDKRRGRDPEMGGKPRRKNPQEGLYNELQKDKMAEAYSEIGMKGERRRGKGHDGLYQGLSTATKDTYDALHMQALPPR

SEQ ID NO: 29 - protein, 27 aa, Homo sapiens
FWVLVVVGGVLACYSLLVTVAFIIFWV

SEQ ID NO: 30 - protein, 41 aa, Homo sapiens
RSKRSRLLHSDYMNMTPRRPGPTRKHYQPYAPPRDFAAYRS

SEQ ID NO: 31 - protein, 251 aa, synthetic construct
  REGION 1..251: note = CD44v6-4GS2, CD44v6-specific single chain fragment
MEAPAQLLFLLLLWLPDTTGEIVLTQSPATLSLSPGERATLSCSASSSINYIYWLQQKPGQAPRILIYLTSNLASGVPARFSGSGSGTDFTLTISSLEPEDFAVYYCLQWSSNPLTFGGGTKVEIKRGGGGSGGGGSEVQLVESGGGLVKPGGSLRLSCAASGFTFSSYDMSWVRQAPGKGLEWVSTISSGGSYTYYLDSIKGRFTISRDNAKNSLYLQMNSLRAEDTAVYYCARQGLDYWGRGTLVTVSS

SEQ ID NO: 32 - protein, 658 aa, synthetic construct
  REGION 1..658: note = CD44v6-4GS2-CAR28z with spacer LNGFR wild-type long (NWL)
MEAPAQLLFLLLLWLPDTTGEIVLTQSPATLSLSPGERATLSCSASSSINYIYWLQQKPGQAPRILIYLTSNLASGVPARFSGSGSGTDFTLTISSLEPEDFAVYYCLQWSSNPLTFGGGTKVEIKRGGGGSGGGGSEVQLVESGGGLVKPGGSLRLSCAASGFTFSSYDMSWVRQAPGKGLEWVSTISSGGSYTYYLDSIKGRFTISRDNAKNSLYLQMNSLRAEDTAVYYCARQGLDYWGRGTLVTVSSGDPKEACPTGLYTHSGECCKACNLGEGVAQPCGANQTVCEPCLDSVTFSDVVSATEPCKPCTECVGLQSMSAPCVEADDAVCRCAYGYYQDETTGRCEACRVCEAGSGLVFSCQDKQNTVCEECPDGTYSDEANHVDPCLPCTVCEDTERQLRECTRWADAECEEIPGRWITRSTPPEGSDSTAPSTQEPEAPPEQDLIASTVAGVVTTVMGSSQPVVTRGTTDNPKFWVLVVVGGVLACYSLLVTVAFIIFWVRSKRSRLLHSDYMNMTPRRPGPTRKHYQPYAPPRDFAAYRSRVKFSRSADAPAYQQGQNQLYNELNLGRREEYDVLDKRRGRDPEMGGKPRRKNPQEGLYNELQKDKMAEAYSEIGMKGERRRGKGHDGLYQGLSTATKDTYDALHMQALPPR

SEQ ID NO: 33 - protein, 598 aa, synthetic construct
  REGION 1..598: note = CD44v6-4GS2-CAR28z with spacer LNGFR wild-type short (NWS)
MEAPAQLLFLLLLWLPDTTGEIVLTQSPATLSLSPGERATLSCSASSSINYIYWLQQKPGQAPRILIYLTSNLASGVPARFSGSGSGTDFTLTISSLEPEDFAVYYCLQWSSNPLTFGGGTKVEIKRGGGGSGGGGSEVQLVESGGGLVKPGGSLRLSCAASGFTFSSYDMSWVRQAPGKGLEWVSTISSGGSYTYYLDSIKGRFTISRDNAKNSLYLQMNSLRAEDTAVYYCARQGLDYWGRGTLVTVSSGDPKEACPTGLYTHSGECCKACNLGEGVAQPCGANQTVCEPCLDSVTFSDVVSATEPCKPCTECVGLQSMSAPCVEADDAVCRCAYGYYQDETTGRCEACRVCEAGSGLVFSCQDKQNTVCEECPDGTYSDEANHVDPCLPCTVCEDTERQLRECTRWADAECEEPKFWVLVVVGGVLACYSLLVTVAFIIFWVRSKRSRLLHSDYMNMTPRRPGPTRKHYQPYAPPRDFAAYRSRVKFSRSADAPAYQQGQNQLYNELNLGRREEYDVLDKRRGRDPEMGGKPRRKNPQEGLYNELQKDKMAEAYSEIGMKGERRRGKGHDGLYQGLSTATKDTYDALHMQALPPR

SEQ ID NO: 34 - protein, 636 aa, synthetic construct
  REGION 1..636: note = CD44v6-4GS2-CAR28z with spacer LNGFR mutated long (NML)
MEAPAQLLFLLLLWLPDTTGEIVLTQSPATLSLSPGERATLSCSASSSINYIYWLQQKPGQAPRILIYLTSNLASGVPARFSGSGSGTDFTLTISSLEPEDFAVYYCLQWSSNPLTFGGGTKVEIKRGGGGSGGGGSEVQLVESGGGLVKPGGSLRLSCAASGFTFSSYDMSWVRQAPGKGLEWVSTISSGGSYTYYLDSIKGRFTISRDNAKNSLYLQMNSLRAEDTAVYYCARQGLDYWGRGTLVTVSSGDPKEACPTGLYTHSGECCKACNLGEGVAQPCGANQTVCEPCLDSVTFSDVVSATEPCKPCTECVGLQSMSAPCVEADDAVCRCAYGYYQDETTGRCEACRVCEAGSGLVFSCQDKQNTVCEECPDGTYSDEAARAADAECEEIPGRWITRSTPPEGSDSTAPSTQEPEAPPEQDLIASTVAGVVTTVMGSSQPVVTRGTTDNPKFWVLVVVGGVLACYSLLVTVAFIIFWVRSKRSRLLHSDYMNMTPRRPGPTRKHYQPYAPPRDFAAYRSRVKFSRSADAPAYQQGQNQLYNELNLGRREEYDVLDKRRGRDPEMGGKPRRKNPQEGLYNELQKDKMAEAYSEIGMKGERRRGKGHDGLYQGLSTATKDTYDALHMQALPPR

SEQ ID NO: 35 - protein, 576 aa, synthetic construct
  REGION 1..576: note = CD44v6-4GS2-CAR28z with spacer LNGFR mutated short (NMS)
MEAPAQLLFLLLLWLPDTTGEIVLTQSPATLSLSPGERATLSCSASSSINYIYWLQQKPGQAPRILIYLTSNLASGVPARFSGSGSGTDFTLTISSLEPEDFAVYYCLQWSSNPLTFGGGTKVEIKRGGGGSGGGGSEVQLVESGGGLVKPGGSLRLSCAASGFTFSSYDMSWVRQAPGKGLEWVSTISSGGSYTYYLDSIKGRFTISRDNAKNSLYLQMNSLRAEDTAVYYCARQGLDYWGRGTLVTVSSGDPKEACPTGLYTHSGECCKACNLGEGVAQPCGANQTVCEPCLDSVTFSDVVSATEPCKPCTECVGLQSMSAPCVEADDAVCRCAYGYYQDETTGRCEACRVCEAGSGLVFSCQDKQNTVCEECPDGTYSDEAARAADAECEEPKFWVLVVVGGVLACYSLLVTVAFIIFWVRSKRSRLLHSDYMNMTPRRPGPTRKHYQPYAPPRDFAAYRSRVKFSRSADAPAYQQGQNQLYNELNLGRREEYDVLDKRRGRDPEMGGKPRRKNPQEGLYNELQKDKMAEAYSEIGMKGERRRGKGHDGLYQGLSTATKDTYDALHMQALPPR

SEQ ID NO: 36 - protein, 10 aa, synthetic construct
  REGION 1..10: note = Peptide linker
GGGGSGGGGS

SEQ ID NO: 37 - DNA, 8331 bp, synthetic construct
  misc_feature 1..8331: note = CD44v6-4GS2-CAR.28Z NGFR WILD TYPE LONG (V6 NWL)
  source 1..8331: mol_type = other DNA
aagctttgctcttaggagtttcctaatacatcccaaactcaaatatataaagcatttgacttgttctatgccctagggggcggggggaagctaagccagctttttttaacatttaaaatgttaattccattttaaatgcacagatgtttttatttcataagggtttcaatgtgcatgaatgctgcaatattcctgttaccaaagctagtataaataaaaatagataaacgtggaaattacttagagtttctgtcattaacgtttccttcctcagttgacaacataaatgcgctgctgagcaagccagtttgcatctgtcaggatcaatttcccattatgccagtcatattaattactagtcaattagttgatttttatttttgacatatacatgtgaatgaaagaccccacctgtaggtttggcaagctagcttaagtaacgccattttgcaaggcatggaaaaatacataactgagaatagaaaagttcagatcaaggtcaggaacagatggaacagctgaatatgggccaaacaggatatctgtggtaagcagttcctgccccggctcagggccaagaacagatggaacagctgaatatgggccaaacaggatatctgtggtaagcagttcctgccccggctcagggccaagaacagatggtccccagatgcggtccagccctcagcagtttctagagaaccatcagatgtttccagggtgccccaaggacctgaaatgaccctgtgccttatttgaactaaccaatcagttcgcttctcgcttctgttcgcgcgcttatgctccccgagctcaataaaagagcccacaacccctcactcggggcgccagtcctccgattgactgagtcgcccgggtacccgtgtatccaataaaccctcttgcagttgcatccgacttgtggtctcgctgttccttgggagggtctcctctgagtgattgactacccgtcagcgggggtctttcatttgggggctcgtccgggatcgggagacccctgcccagggaccaccgacccaccaccgggaggtaagctggccagcaacttatctgtgtctgtccgattgtctagtgtctatgactgattttatgcgcctgcgtcggtactagttagctaactagctctgtatctggcggacccgtggtggaactgacgagttcggaacacccggccgcaaccctgggagacgtcccagggacttcgggggccgtttttgtggcccgacctgagtcctaaaatcccgatcgtttaggactctttggtgcaccccccttagaggagggatatgtggttctggtaggagacgagaacctaaaacagttcccgcctccgtctgaatttttgctttcggtttgggaccgaagccgcgccgcgcgtcttgtctgctgcagcatcgttctgtgttgtctctgtctgactgtgtttctgtatttgtctgaaaatatgggcccgggctagcctgttaccactcccttaagtttgaccttaggtcactggaaagatgtcgagcggatcgctcacaaccagtcggtagatgtcaagaagagacgttgggttaccttctgctctgcagaatggccaacctttaacgtcggatggccgcgagacggcacctttaaccgagacctcatcacccaggttaagatcaaggtcttttcacctggcccgcatggacacccagaccaggtggggtacatcgtgacctgggaagccttggcttttgacccccctccctgggtcaagccctttgtacaccctaagcctccgcctcctcttcctccatccgccccgtctctcccccttgaacctcctcgttcgaccccgcctcgatcctccctttatccagccctcactccttctctaggcgcccccatatggccatatgagatcttatatggggcacccccgccccttgtaaacttccctgaccctgacatgacaagagttactaacagcccctctctccaagctcacttacaggctctctacttagtccagcacgaagtctggagacctctggcggcagcctaccaagaacaactggaccgaccggtggtacctcacccttaccgagtcggcgacacagtgtgggtccgccgacaccagactaagaacctagaacctcgctggaaaggaccttacacagtcctgctgaccacccccaccgccctcaaagtagacggcatcgcagcttggatacacgccgcccacgtgaaggctgccgaccccgggggtggaccatcctctagactgccatggaagcccctgcccagctgctgttcctgctgctgctgtggctgcccgacaccaccggcgagatcgtgctgacacagagccccgccaccctgtctctgagccctggcgagagagccaccctgagctgtagcgccagcagcagcatcaactacatctactggctgcagcagaagcccggccaggcccccagaatcctgatctacctgaccagcaacctggccagcggcgtgcccgccagattttctggcagcggcagcggcaccgacttcaccctgaccatcagcagcctggaacccgaggacttcgccgtgtactactgcctgcagtggtccagcaaccccctgaccttcggcggaggcaccaaggtggaaatcaagcggggtggtggtggttctggtggtggtggttctgaggtgcagctggtggaaagcggcggaggcctggtcaagcctggcggcagcctgagactgagctgtgccgccagcggcttcaccttcagcagctacgacatgagctgggtccgacaggctccaggcaagggactggaatgggtgtccaccatcagcagcggcggcagctacacctactacctggacagcatcaagggccggttcaccatcagccgggacaacgccaagaacagcctgtacctgcagatgaacagcctgcgggccgaggacaccgccgtctactactgtgcccggcagggcctcgactactggggcagaggcaccctggtcaccgtgtccagcggggatcccaaagaggcctgccccaccggcctgtacacccacagcggagagtgctgcaaggcctgcaacctgggagagggcgtggcccagccttgcggcgccaatcagaccgtgtgcgagccctgcctggacagcgtgaccttcagcgacgtggtgtccgccaccgagccctgcaagccttgcaccgagtgtgtgggcctgcagagcatgagcgccccctgcgtggaagccgacgacgccgtgtgtagatgcgcctacggctactaccaggacgagacaaccggcagatgcgaggcctgtagagtgtgcgaggccggcagcggcctggtgttcagttgtcaagacaagcagaataccgtgtgtgaagagtgccccgacggcacctacagcgacgaggccaaccacgtggacccctgcctgccctgcactgtgtgcgaggacaccgagcggcagctgcgcgagtgcacaagatgggccgacgccgagtgcgaagagatccccggcagatggatcaccagaagcaccccccctgagggcagcgacagcaccgcccctagcacccaggaacctgaggcccctcccgagcaggacctgatcgcctctacagtggccggcgtggtgacaaccgtgatgggcagctctcagcccgtggtgacacggggcaccaccgacaatcccaaattttgggtgctggtggtggttggtggagtcctggcttgctatagcttgctagtaacagtggcctttattattttctgggtgaggagtaagaggagcaggctcctgcacagtgactacatgaacatgactccccgccgccccgggcccacccgcaagcattaccagccctatgccccaccacgcgacttcgcagcctatcgctccagagtgaagttcagcaggagcgcagacgcccccgcgtaccagcagggccagaaccagctctataacgagctcaatctaggacgaagagaggagtacgatgttttggacaagagacgtggccgggaccctgagatggggggaaagccgagaaggaagaaccctcaggaaggcctgtacaatgaactgcagaaagataagatggcggaggcctacagtgagattgggatgaaaggcgagcgccggaggggcaaggggcacgatggcctttaccagggtctcagtacagccaccaaggacacctacgacgcccttcacatgcaggccctgcctcctcgctaagcatgcaacctcgatccggattagtccaatttgttaaagacaggatatcagtggtccaggctctagttttgactcaacaatatcaccagctgaagcctatagagtacgagccatagataaaataaaagattttatttagtctccagaaaaaggggggaatgaaagaccccacctgtaggtttggcaagctagcttaagtaacgccattttgcaaggcatggaaaaatacataactgagaatagagaagttcagatcaaggtcaggaacagatggaacagctgaatatgggccaaacaggatatctgtggtaagcagttcctgccccggctcagggccaagaacagatggaacagctgaatatgggccaaacaggatatctgtggtaagcagttcctgccccggctcagggccaagaacagatggtccccagatgcggtccagccctcagcagtttctagagaaccatcagatgtttccagggtgccccaaggacctgaaatgaccctgtgccttatttgaactaaccaatcagttcgcttctcgcttctgttcgcgcgcttctgctccccgagctcaataaaagagcccacaacccctcactcggggcgccagtcctccgattgactgagtcgcccgggtacccgtgtatccaataaaccctcttgcagttgcatccgacttgtggtctcgctgttccttgggagggtctcctctgagtgattgactacccgtcagcgggggtctttcacacatgcagcatgtatcaaaattaatttggttttttttcttaagtatttacattaaatggccatagtacttaaagttacattggcttccttgaaataaacatggagtattcagaatgtgtcataaatatttctaattttaagatagtatctccattggctttctactttttcttttatttttttttgtcctctgtcttccatttgttgttgttgttgtttgtttgtttgtttgttggttggttggttaatttttttttaaagatcctacactatagttcaagctagactattagctactctgtaacccagggtgaccttgaagtcatgggtagcctgctgttttagccttcccacatctaagattacaggtatgagctatcatttttggtatattgattgattgattgattgatgtgtgtgtgtgtgattgtgtttgtgtgtgtgactgtgaaaatgtgtgtatgggtgtgtgtgaatgtgtgtatgtatgtgtgtgtgtgagtgtgtgtgtgtgtgtgtgcatgtgtgtgtgtgtgactgtgtctatgtgtatgactgtgtgtgtgtgtgtgtgtgtgtgtgtgtgtgtgtgtgtgtgtgtgttgtgaaaaaatattctatggtagtgagagccaacgctccggctcaggtgtcaggttggtttttgagacagagtctttcacttagcttggaattcactggccgtcgttttacaacgtcgtgactgggaaaaccctggcgttacccaacttaatcgccttgcagcacatccccctttcgccagctggcgtaatagcgaagaggcccgcaccgatcgcccttcccaacagttgcgcagcctgaatggcgaatggcgcctgatgcggtattttctccttacgcatctgtgcggtatttcacaccgcatatggtgcactctcagtacaatctgctctgatgccgcatagttaagccagccccgacacccgccaacacccgctgacgcgccctgacgggcttgtctgctcccggcatccgcttacagacaagctgtgaccgtctccgggagctgcatgtgtcagaggttttcaccgtcatcaccgaaacgcgcgatgacgaaagggcctcgtgatacgcctatttttataggttaatgtcatgataataatggtttcttagacgtcaggtggcacttttcggggaaatgtgcgcggaacccctatttgtttatttttctaaatacattcaaatatgtatccgctcatgagacaataaccctgataaatgcttcaataatattgaaaaaggaagagtatgagtattcaacatttccgtgtcgcccttattcccttttttgcggcattttgccttcctgtttttgctcacccagaaacgctggtgaaagtaaaagatgctgaagatcagttgggtgcacgagtgggttacatcgaactggatctcaacagcggtaagatccttgagagttttcgccccgaagaacgttttccaatgatgagcacttttaaagttctgctatgtggcgcggtattatcccgtattgacgccgggcaagagcaactcggtcgccgcatacactattctcagaatgacttggttgagtactcaccagtcacagaaaagcatcttacggatggcatgacagtaagagaattatgcagtgctgccataaccatgagtgataacactgcggccaacttacttctgacaacgatcggaggaccgaaggagctaaccgcttttttgcacaacatgggggatcatgtaactcgccttgatcgttgggaaccggagctgaatgaagccataccaaacgacgagcgtgacaccacgatgcctgtagcaatggcaacaacgttgcgcaaactattaactggcgaactacttactctagcttcccggcaacaattaatagactggatggaggcggataaagttgcaggaccacttctgcgctcggcccttccggctggctggtttattgctgataaatctggagccggtgagcgtgggtctcgcggtatcattgcagcactggggccagatggtaagccctcccgtatcgtagttatctacacgacggggagtcaggcaactatggatgaacgaaatagacagatcgctgagataggtgcctcactgattaagcattggtaactgtcagaccaagtttactcatatatactttagattgatttaaaacttcatttttaatttaaaaggatctaggtgaagatcctttttgataatctcatgaccaaaatcccttaacgtgagttttcgttccactgagcgtcagaccccgtagaaaagatcaaaggatcttcttgagatcctttttttctgcgcgtaatctgctgcttgcaaacaaaaaaaccaccgctaccagcggtggtttgtttgccggatcaagagctaccaactctttttccgaaggtaactggcttcagcagagcgcagataccaaatactgtccttctagtgtagccgtagttaggccaccacttcaagaactctgtagcaccgcctacatacctcgctctgctaatcctgttaccagtggctgctgccagtggcgataagtcgtgtcttaccgggttggactcaagacgatagttaccggataaggcgcagcggtcgggctgaacggggggttcgtgcacacagcccagcttggagcgaacgacctacaccgaactgagatacctacagcgtgagcattgagaaagcgccacgcttcccgaagggagaaaggcggacaggtatccggtaagcggcagggtcggaacaggagagcgcacgagggagcttccagggggaaacgcctggtatctttatagtcctgtcgggtttcgccacctctgacttgagcgtcgatttttgtgatgctcgtcaggggggcggagcctatggaaaaacgccagcaacgcggcctttttacggttcctggccttttgctggccttttgctcacatgttctttcctgcgttatcccctgattctgtggataaccgtattaccgcctttgagtgagctgataccgctcgccgcagccgaacgaccgagcgcagcgagtcagtgagcgaggaagcggaagagcgcccaatacgcaaaccgcctctccccgcgcgttggccgattcattaatgcagctggcacgacaggtttcccgactggaaagcgggcagtgagcgcaacgcaattaatgtgagttagctcactcattaggcaccccaggctttacactttatgcttccggctcgtatgttgtgtggaattgtgagcggataacaatttcacacaggaaacagctatgaccatgattacgcc

SEQ ID NO: 38 - DNA, 8151 bp, synthetic construct
  misc_feature 1..8151: note = CD44V6-4GS2-CAR.28Z NGFR WILD TYPE SHORT (V6 NWS)
  source 1..8151: mol_type = other DNA
aagctttgctcttaggagtttcctaatacatcccaaactcaaatatataaagcatttgacttgttctatgccctagggggcggggggaagctaagccagctttttttaacatttaaaatgttaattccattttaaatgcacagatgtttttatttcataagggtttcaatgtgcatgaatgctgcaatattcctgttaccaaagctagtataaataaaaatagataaacgtggaaattacttagagtttctgtcattaacgtttccttcctcagttgacaacataaatgcgctgctgagcaagccagtttgcatctgtcaggatcaatttcccattatgccagtcatattaattactagtcaattagttgatttttatttttgacatatacatgtgaatgaaagaccccacctgtaggtttggcaagctagcttaagtaacgccattttgcaaggcatggaaaaatacataactgagaatagaaaagttcagatcaaggtcaggaacagatggaacagctgaatatgggccaaacaggatatctgtggtaagcagttcctgccccggctcagggccaagaacagatggaacagctgaatatgggccaaacaggatatctgtggtaagcagttcctgccccggctcagggccaagaacagatggtccccagatgcggtccagccctcagcagtttctagagaaccatcagatgtttccagggtgccccaaggacctgaaatgaccctgtgccttatttgaactaaccaatcagttcgcttctcgcttctgttcgcgcgcttatgctccccgagctcaataaaagagcccacaacccctcactcggggcgccagtcctccgattgactgagtcgcccgggtacccgtgtatccaataaaccctcttgcagttgcatccgacttgtggtctcgctgttccttgggagggtctcctctgagtgattgactacccgtcagcgggggtctttcatttgggggctcgtccgggatcgggagacccctgcccagggaccaccgacccaccaccgggaggtaagctggccagcaacttatctgtgtctgtccgattgtctagtgtctatgactgattttatgcgcctgcgtcggtactagttagctaactagctctgtatctggcggacccgtggtggaactgacgagttcggaacacccggccgcaaccctgggagacgtcccagggacttcgggggccgtttttgtggcccgacctgagtcctaaaatcccgatcgtttaggactctttggtgcaccccccttagaggagggatatgtggttctggtaggagacgagaacctaaaacagttcccgcctccgtctgaatttttgctttcggtttgggaccgaagccgcgccgcgcgtcttgtctgctgcagcatcgttctgtgttgtctctgtctgactgtgtttctgtatttgtctgaaaatatgggcccgggctagcctgttaccactcccttaagtttgaccttaggtcactggaaagatgtcgagcggatcgctcacaaccagtcggtagatgtcaagaagagacgttgggttaccttctgctctgcagaatggccaacctttaacgtcggatggccgcgagacggcacctttaaccgagacctcatcacccaggttaagatcaaggtcttttcacctggcccgcatggacacccagaccaggtggggtacatcgtgacctgggaagccttggcttttgacccccctccctgggtcaagccctttgtacaccctaagcctccgcctcctcttcctccatccgccccgtctctcccccttgaacctcctcgttcgaccccgcctcgatcctccctttatccagccctcactccttctctaggcgcccccatatggccatatgagatcttatatggggcacccccgccccttgtaaacttccctgaccctgacatgacaagagttactaacagcccctctctccaagctcacttacaggctctctacttagtccagcacgaagtctggagacctctggcggcagcctaccaagaacaactggaccgaccggtggtacctcacccttaccgagtcggcgacacagtgtgggtccgccgacaccagactaagaacctagaacctcgctggaaaggaccttacacagtcctgctgaccacccccaccgccctcaaagtagacggcatcgcagcttggatacacgccgcccacgtgaaggctgccgaccccgggggtggaccatcctctagactgccatggaagcccctgcccagctgctgttcctgctgctgctgtggctgcccgacaccaccggcgagatcgtgctgacacagagccccgccaccctgtctctgagccctggcgagagagccaccctgagctgtagcgccagcagcagcatcaactacatctactggctgcagcagaagcccggccaggcccccagaatcctgatctacctgaccagcaacctggccagcggcgtgcccgccagattttctggcagcggcagcggcaccgacttcaccctgaccatcagcagcctggaacccgaggacttcgccgtgtactactgcctgcagtggtccagcaaccccctgaccttcggcggaggcaccaaggtggaaatcaagcggggtggtggtggttctggtggtggtggttctgaggtgcagctggtggaaagcggcggaggcctggtcaagcctggcggcagcctgagactgagctgtgccgccagcggcttcaccttcagcagctacgacatgagctgggtccgacaggctccaggcaagggactggaatgggtgtccaccatcagcagcggcggcagctacacctactacctggacagcatcaagggccggttcaccatcagccgggacaacgccaagaacagcctgtacctgcagatgaacagcctgcgggccgaggacaccgccgtctactactgtgcccggcagggcctcgactactggggcagaggcaccctggtcaccgtgtccagcggggatcccaaagaggcctgccccaccggcctgtacacccacagcggagagtgctgcaaggcctgcaacctgggagagggcgtggcccagccttgcggcgccaatcagaccgtgtgcgagccctgcctggacagcgtgaccttcagcgacgtggtgtccgccaccgagccctgcaagccttgcaccgagtgtgtgggcctgcagagcatgagcgccccctgcgtggaagccgacgacgccgtgtgtagatgcgcctacggctactaccaggacgagacaaccggcagatgcgaggcctgtagagtgtgcgaggccggcagcggcctggtgttcagttgtcaggacaagcagaacaccgtgtgtgaagagtgccccgacggcacctacagcgacgaggccaaccacgtggacccctgcctgccctgcactgtgtgcgaggacaccgagcggcagctgcgcgagtgcacaagatgggccgacgccgagtgcgaggaacccaaattttgggtgctggtggtggttggtggagtcctggcttgctatagcttgctagtaacagtggcctttattattttctgggtgaggagtaagaggagcaggctcctgcacagtgactacatgaacatgactccccgccgccccgggcccacccgcaagcattaccagccctatgccccaccacgcgacttcgcagcctatcgctccagagtgaagttcagcaggagcgcagacgcccccgcgtaccagcagggccagaaccagctctataacgagctcaatctaggacgaagagaggagtacgatgttttggacaagagacgtggccgggaccctgagatggggggaaagccgagaaggaagaaccctcaggaaggcctgtacaatgaactgcagaaagataagatggcggaggcctacagtgagattgggatgaaaggcgagcgccggaggggcaaggggcacgatggcctttaccagggtctcagtacagccaccaaggacacctacgacgcccttcacatgcaggccctgcctcctcgctaagcatgcaacctcgatccggattagtccaatttgttaaagacaggatatcagtggtccaggctctagttttgactcaacaatatcaccagctgaagcctatagagtacgagccatagataaaataaaagattttatttagtctccagaaaaaggggggaatgaaagaccccacctgtaggtttggcaagctagcttaagtaacgccattttgcaaggcatggaaaaatacataactgagaatagagaagttcagatcaaggtcaggaacagatggaacagctgaatatgggccaaacaggatatctgtggtaagcagttcctgccccggctcagggccaagaacagatggaacagctgaatatgggccaaacaggatatctgtggtaagcagttcctgccccggctcagggccaagaacagatggtccccagatgcggtccagccctcagcagtttctagagaaccatcagatgtttccagggtgccccaaggacctgaaatgaccctgtgccttatttgaactaaccaatcagttcgcttctcgcttctgttcgcgcgcttctgctccccgagctcaataaaagagcccacaacccctcactcggggcgccagtcctccgattgactgagtcgcccgggtacccgtgtatccaataaaccctcttgcagttgcatccgacttgtggtctcgctgttccttgggagggtctcctctgagtgattgactacccgtcagcgggggtctttcacacatgcagcatgtatcaaaattaatttggttttttttcttaagtatttacattaaatggccatagtacttaaagttacattggcttccttgaaataaacatggagtattcagaatgtgtcataaatatttctaattttaagatagtatctccattggctttctactttttcttttatttttttttgtcctctgtcttccatttgttgttgttgttgtttgtttgtttgtttgttggttggttggttaatttttttttaaagatcctacactatagttcaagctagactattagctactctgtaacccagggtgaccttgaagtcatgggtagcctgctgttttagccttcccacatctaagattacaggtatgagctatcatttttggtatattgattgattgattgattgatgtgtgtgtgtgtgattgtgtttgtgtgtgtgactgtgaaaatgtgtgtatgggtgtgtgtgaatgtgtgtatgtatgtgtgtgtgtgagtgtgtgtgtgtgtgtgtgcatgtgtgtgtgtgtgactgtgtctatgtgtatgactgtgtgtgtgtgtgtgtgtgtgtgtgtgtgtgtgtgtgtgtgtgtgttgtgaaaaaatattctatggtagtgagagccaacgctccggctcaggtgtcaggttggtttttgagacagagtctttcacttagcttggaattcactggccgtcgttttacaacgtcgtgactgggaaaaccctggcgttacccaacttaatcgccttgcagcacatccccctttcgccagctggcgtaatagcgaagaggcccgcaccgatcgcccttcccaacagttgcgcagcctgaatggcgaatggcgcctgatgcggtattttctccttacgcatctgtgcggtatttcacaccgcatatggtgcactctcagtacaatctgctctgatgccgcatagttaagccagccccgacacccgccaacacccgctgacgcgccctgacgggcttgtctgctcccggcatccgcttacagacaagctgtgaccgtctccgggagctgcatgtgtcagaggttttcaccgtcatcaccgaaacgcgcgatgacgaaagggcctcgtgatacgcctatttttataggttaatgtcatgataataatggtttcttagacgtcaggtggcacttttcggggaaatgtgcgcggaacccctatttgtttatttttctaaatacattcaaatatgtatccgctcatgagacaataaccctgataaatgcttcaataatattgaaaaaggaagagtatgagtattcaacatttccgtgtcgcccttattcccttttttgcggcattttgccttcctgtttttgctcacccagaaacgctggtgaaagtaaaagatgctgaagatcagttgggtgcacgagtgggttacatcgaactggatctcaacagcggtaagatccttgagagttttcgccccgaagaacgttttccaatgatgagcacttttaaagttctgctatgtggcgcggtattatcccgtattgacgccgggcaagagcaactcggtcgccgcatacactattctcagaatgacttggttgagtactcaccagtcacagaaaagcatcttacggatggcatgacagtaagagaattatgcagtgctgccataaccatgagtgataacactgcggccaacttacttctgacaacgatcggaggaccgaaggagctaaccgcttttttgcacaacatgggggatcatgtaactcgccttgatcgttgggaaccggagctgaatgaagccataccaaacgacgagcgtgacaccacgatgcctgtagcaatggcaacaacgttgcgcaaactattaactggcgaactacttactctagcttcccggcaacaattaatagactggatggaggcggataaagttgcaggaccacttctgcgctcggcccttccggctggctggtttattgctgataaatctggagccggtgagcgtgggtctcgcggtatcattgcagcactggggccagatggtaagccctcccgtatcgtagttatctacacgacggggagtcaggcaactatggatgaacgaaatagacagatcgctgagataggtgcctcactgattaagcattggtaactgtcagaccaagtttactcatatatactttagattgatttaaaacttcatttttaatttaaaaggatctaggtgaagatcctttttgataatctcatgaccaaaatcccttaacgtgagttttcgttccactgagcgtcagaccccgtagaaaagatcaaaggatcttcttgagatcctttttttctgcgcgtaatctgctgcttgcaaacaaaaaaaccaccgctaccagcggtggtttgtttgccggatcaagagctaccaactctttttccgaaggtaactggcttcagcagagcgcagataccaaatactgtccttctagtgtagccgtagttaggccaccacttcaagaactctgtagcaccgcctacatacctcgctctgctaatcctgttaccagtggctgctgccagtggcgataagtcgtgtcttaccgggttggactcaagacgatagttaccggataaggcgcagcggtcgggctgaacggggggttcgtgcacacagcccagcttggagcgaacgacctacaccgaactgagatacctacagcgtgagcattgagaaagcgccacgcttcccgaagggagaaaggcggacaggtatccggtaagcggcagggtcggaacaggagagcgcacgagggagcttccagggggaaacgcctggtatctttatagtcctgtcgggtttcgccacctctgacttgagcgtcgatttttgtgatgctcgtcaggggggcggagcctatggaaaaacgccagcaacgcggcctttttacggttcctggccttttgctggccttttgctcacatgttctttcctgcgttatcccctgattctgtggataaccgtattaccgcctttgagtgagctgataccgctcgccgcagccgaacgaccgagcgcagcgagtcagtgagcgaggaagcggaagagcgcccaatacgcaaaccgcctctccccgcgcgttggccgattcattaatgcagctggcacgacaggtttcccgactggaaagcgggcagtgagcgcaacgcaattaatgtgagttagctcactcattaggcaccccaggctttacactttatgcttccggctcgtatgttgtgtggaattgtgagcggataacaatttcacacaggaaacagctatgaccatgattacgcc

SEQ ID NO: 39 - DNA, 8265 bp, synthetic construct
  misc_feature 1..8265: note = CD44v6-4GS2-CAR.28Z NGFR MUTATED LONG (V6 NML)
  source 1..8265: mol_type = other DNA
aagctttgctcttaggagtttcctaatacatcccaaactcaaatatataaagcatttgacttgttctatgccctagggggcggggggaagctaagccagctttttttaacatttaaaatgttaattccattttaaatgcacagatgtttttatttcataagggtttcaatgtgcatgaatgctgcaatattcctgttaccaaagctagtataaataaaaatagataaacgtggaaattacttagagtttctgtcattaacgtttccttcctcagttgacaacataaatgcgctgctgagcaagccagtttgcatctgtcaggatcaatttcccattatgccagtcatattaattactagtcaattagttgatttttatttttgacatatacatgtgaatgaaagaccccacctgtaggtttggcaagctagcttaagtaacgccattttgcaaggcatggaaaaatacataactgagaatagaaaagttcagatcaaggtcaggaacagatggaacagctgaatatgggccaaacaggatatctgtggtaagcagttcctgccccggctcagggccaagaacagatggaacagctgaatatgggccaaacaggatatctgtggtaagcagttcctgccccggctcagggccaagaacagatggtccccagatgcggtccagccctcagcagtttctagagaaccatcagatgtttccagggtgccccaaggacctgaaatgaccctgtgccttatttgaactaaccaatcagttcgcttctcgcttctgttcgcgcgcttatgctccccgagctcaataaaagagcccacaacccctcactcggggcgccagtcctccgattgactgagtcgcccgggtacccgtgtatccaataaaccctcttgcagttgcatccgacttgtggtctcgctgttccttgggagggtctcctctgagtgattgactacccgtcagcgggggtctttcatttgggggctcgtccgggatcgggagacccctgcccagggaccaccgacccaccaccgggaggtaagctggccagcaacttatctgtgtctgtccgattgtctagtgtctatgactgattttatgcgcctgcgtcggtactagttagctaactagctctgtatctggcggacccgtggtggaactgacgagttcggaacacccggccgcaaccctgggagacgtcccagggacttcgggggccgtttttgtggcccgacctgagtcctaaaatcccgatcgtttaggactctttggtgcaccccccttagaggagggatatgtggttctggtaggagacgagaacctaaaacagttcccgcctccgtctgaatttttgctttcggtttgggaccgaagccgcgccgcgcgtcttgtctgctgcagcatcgttctgtgttgtctctgtctgactgtgtttctgtatttgtctgaaaatatgggcccgggctagcctgttaccactcccttaagtttgaccttaggtcactggaaagatgtcgagcggatcgctcacaaccagtcggtagatgtcaagaagagacgttgggttaccttctgctctgcagaatggccaacctttaacgtcggatggccgcgagacggcacctttaaccgagacctcatcacccaggttaagatcaaggtcttttcacctggcccgcatggacacccagaccaggtggggtacatcgtgacctgggaagccttggcttttgacccccctccctgggtcaagccctttgtacaccctaagcctccgcctcctcttcctccatccgccccgtctctcccccttgaacctcctcgttcgaccccgcctcgatcctccctttatccagccctcactccttctctaggcgcccccatatggccatatgagatcttatatggggcacccccgccccttgtaaacttccctgaccctgacatgacaagagttactaacagcccctctctccaagctcacttacaggctctctacttagtccagcacgaagtctggagacctctggcggcagcctaccaagaacaactggaccgaccggtggtacctcacccttaccgagtcggcgacacagtgtgggtccgccgacaccagactaagaacctagaacctcgctggaaaggaccttacacagtcctgctgaccacccccaccgccctcaaagtagacggcatcgcagcttggatacacgccgcccacgtgaaggctgccgaccccgggggtggaccatcctctagactgccatggaagcccctgcccagctgctgttcctgctgctgctgtggctgcccgacaccaccggcgagatcgtgctgacacagagccccgccaccctgtctctgagccctggcgagagagccaccctgagctgtagcgccagcagcagcatcaactacatctactggctgcagcagaagcccggccaggcccccagaatcctgatctacctgaccagcaacctggccagcggcgtgcccgccagattttctggcagcggcagcggcaccgacttcaccctgaccatcagcagcctggaacccgaggacttcgccgtgtactactgcctgcagtggtccagcaaccccctgaccttcggcggaggcaccaaggtggaaatcaagcggggtggtggtggttctggtggtggtggttctgaggtgcagctggtggaaagcggcggaggcctggtcaagcctggcggcagcctgagactgagctgtgccgccagcggcttcaccttcagcagctacgacatgagctgggtccgacaggctccaggcaagggactggaatgggtgtccaccatcagcagcggcggcagctacacctactacctggacagcatcaagggccggttcaccatcagccgggacaacgccaagaacagcctgtacctgcagatgaacagcctgcgggccgaggacaccgccgtctactactgtgcccggcagggcctcgactactggggcagaggcaccctggtcaccgtgtccagcggggatcccaaagaggcctgccccaccggcctgtacacccacagcggagagtgctgcaaggcctgcaacctgggagagggcgtggcccagccttgcggcgccaatcagaccgtgtgcgagccctgcctggacagcgtgaccttcagcgacgtggtgtccgccaccgagccctgcaagccttgcaccgagtgtgtgggcctgcagagcatgagcgccccctgcgtggaagccgacgacgccgtgtgtagatgcgcctacggctactaccaggacgagacaaccggcagatgcgaggcctgtagagtgtgcgaggccggcagcggcctggtgttcagttgtcaagacaagcagaataccgtgtgtgaagagtgccccgacggcacctacagcgacgaagccgccagagccgccgacgccgagtgcgaagagatccccggcagatggatcaccagaagcaccccccctgagggcagcgacagcaccgcccctagcacccaggaacctgaggcccctcccgagcaggacctgatcgcctctacagtggccggcgtggtgacaaccgtgatgggcagctctcagcccgtggtgacacggggcaccaccgacaatcccaaattttgggtgctggtggtggttggtggagtcctggcttgctatagcttgctagtaacagtggcctttattattttctgggtgaggagtaagaggagcaggctcctgcacagtgactacatgaacatgactccccgccgccccgggcccacccgcaagcattaccagccctatgccccaccacgcgacttcgcagcctatcgctccagagtgaagttcagcaggagcgcagacgcccccgcgtaccagcagggccagaaccagctctataacgagctcaatctaggacgaagagaggagtacgatgttttggacaagagacgtggccgggaccctgagatggggggaaagccgagaaggaagaaccctcaggaaggcctgtacaatgaactgcagaaagataagatggcggaggcctacagtgagattgggatgaaaggcgagcgccggaggggcaaggggcacgatggcctttaccagggtctcagtacagccaccaaggacacctacgacgcccttcacatgcaggccctgcctcctcgctaagcatgcaacctcgatccggattagtccaatttgttaaagacaggatatcagtggtccaggctctagttttgactcaacaatatcaccagctgaagcctatagagtacgagccatagataaaataaaagattttatttagtctccagaaaaaggggggaatgaaagaccccacctgtaggtttggcaagctagcttaagtaacgccattttgcaaggcatggaaaaatacataactgagaatagagaagttcagatcaaggtcaggaacagatggaacagctgaatatgggccaaacaggatatctgtggtaagcagttcctgccccggctcagggccaagaacagatggaacagctgaatatgggccaaacaggatatctgtggtaagcagttcctgccccggctcagggccaagaacagatggtccccagatgcggtccagccctcagcagtttctagagaaccatcagatgtttccagggtgccccaaggacctgaaatgaccctgtgccttatttgaactaaccaatcagttcgcttctcgcttctgttcgcgcgcttctgctccccgagctcaataaaagagcccacaacccctcactcggggcgccagtcctccgattgactgagtcgcccgggtacccgtgtatccaataaaccctcttgcagttgcatccgacttgtggtctcgctgttccttgggagggtctcctctgagtgattgactacccgtcagcgggggtctttcacacatgcagcatgtatcaaaattaatttggttttttttcttaagtatttacattaaatggccatagtacttaaagttacattggcttccttgaaataaacatggagtattcagaatgtgtcataaatatttctaattttaagatagtatctccattggctttctactttttcttttatttttttttgtcctctgtcttccatttgttgttgttgttgtttgtttgtttgtttgttggttggttggttaatttttttttaaagatcctacactatagttcaagctagactattagctactctgtaacccagggtgaccttgaagtcatgggtagcctgctgttttagccttcccacatctaagattacaggtatgagctatcatttttggtatattgattgattgattgattgatgtgtgtgtgtgtgattgtgtttgtgtgtgtgactgtgaaaatgtgtgtatgggtgtgtgtgaatgtgtgtatgtatgtgtgtgtgtgagtgtgtgtgtgtgtgtgtgcatgtgtgtgtgtgtgactgtgtctatgtgtatgactgtgtgtgtgtgtgtgtgtgtgtgtgtgtgtgtgtgtgtgtgtgtgttgtgaaaaaatattctatggtagtgagagccaacgctccggctcaggtgtcaggttggtttttgagacagagtctttcacttagcttggaattcactggccgtcgttttacaacgtcgtgactgggaaaaccctggcgttacccaacttaatcgccttgcagcacatccccctttcgccagctggcgtaatagcgaagaggcccgcaccgatcgcccttcccaacagttgcgcagcctgaatggcgaatggcgcctgatgcggtattttctccttacgcatctgtgcggtatttcacaccgcatatggtgcactctcagtacaatctgctctgatgccgcatagttaagccagccccgacacccgccaacacccgctgacgcgccctgacgggcttgtctgctcccggcatccgcttacagacaagctgtgaccgtctccgggagctgcatgtgtcagaggttttcaccgtcatcaccgaaacgcgcgatgacgaaagggcctcgtgatacgcctatttttataggttaatgtcatgataataatggtttcttagacgtcaggtggcacttttcggggaaatgtgcgcggaacccctatttgtttatttttctaaatacattcaaatatgtatccgctcatgagacaataaccctgataaatgcttcaataatattgaaaaaggaagagtatgagtattcaacatttccgtgtcgcccttattcccttttttgcggcattttgccttcctgtttttgctcacccagaaacgctggtgaaagtaaaagatgctgaagatcagttgggtgcacgagtgggttacatcgaactggatctcaacagcggtaagatccttgagagttttcgccccgaagaacgttttccaatgatgagcacttttaaagttctgctatgtggcgcggtattatcccgtattgacgccgggcaagagcaactcggtcgccgcatacactattctcagaatgacttggttgagtactcaccagtcacagaaaagcatcttacggatggcatgacagtaagagaattatgcagtgctgccataaccatgagtgataacactgcggccaacttacttctgacaacgatcggaggaccgaaggagctaaccgcttttttgcacaacatgggggatcatgtaactcgccttgatcgttgggaaccggagctgaatgaagccataccaaacgacgagcgtgacaccacgatgcctgtagcaatggcaacaacgttgcgcaaactattaactggcgaactacttactctagcttcccggcaacaattaatagactggatggaggcggataaagttgcaggaccacttctgcgctcggcccttccggctggctggtttattgctgataaatctggagccggtgagcgtgggtctcgcggtatcattgcagcactggggccagatggtaagccctcccgtatcgtagttatctacacgacggggagtcaggcaactatggatgaacgaaatagacagatcgctgagataggtgcctcactgattaagcattggtaactgtcagaccaagtttactcatatatactttagattgatttaaaacttcatttttaatttaaaaggatctaggtgaagatcctttttgataatctcatgaccaaaatcccttaacgtgagttttcgttccactgagcgtcagaccccgtagaaaagatcaaaggatcttcttgagatcctttttttctgcgcgtaatctgctgcttgcaaacaaaaaaaccaccgctaccagcggtggtttgtttgccggatcaagagctaccaactctttttccgaaggtaactggcttcagcagagcgcagataccaaatactgtccttctagtgtagccgtagttaggccaccacttcaagaactctgtagcaccgcctacatacctcgctctgctaatcctgttaccagtggctgctgccagtggcgataagtcgtgtcttaccgggttggactcaagacgatagttaccggataaggcgcagcggtcgggctgaacggggggttcgtgcacacagcccagcttggagcgaacgacctacaccgaactgagatacctacagcgtgagcattgagaaagcgccacgcttcccgaagggagaaaggcggacaggtatccggtaagcggcagggtcggaacaggagagcgcacgagggagcttccagggggaaacgcctggtatctttatagtcctgtcgggtttcgccacctctgacttgagcgtcgatttttgtgatgctcgtcaggggggcggagcctatggaaaaacgccagcaacgcggcctttttacggttcctggccttttgctggccttttgctcacatgttctttcctgcgttatcccctgattctgtggataaccgtattaccgcctttgagtgagctgataccgctcgccgcagccgaacgaccgagcgcagcgagtcagtgagcgaggaagcggaagagcgcccaatacgcaaaccgcctctccccgcgcgttggccgattcattaatgcagctggcacgacaggtttcccgactggaaagcgggcagtgagcgcaacgcaattaatgtgagttagctcactcattaggcaccccaggctttacactttatgcttccggctcgtatgttgtgtggaattgtgagcggataacaatttcacacaggaaacagctatgaccatgattacgcc

SEQ ID NO: 40 - DNA, 8085 bp, synthetic construct
  misc_feature 1..8085: note = CD44v6-4GS2-CAR.28Z NGFR MUTATED SHORT (V6 NMS)
  source 1..8085: mol_type = other DNA
aagctttgctcttaggagtttcctaatacatcccaaactcaaatatataaagcatttgacttgttctatgccctagggggcggggggaagctaagccagctttttttaacatttaaaatgttaattccattttaaatgcacagatgtttttatttcataagggtttcaatgtgcatgaatgctgcaatattcctgttaccaaagctagtataaataaaaatagataaacgtggaaattacttagagtttctgtcattaacgtttccttcctcagttgacaacataaatgcgctgctgagcaagccagtttgcatctgtcaggatcaatttcccattatgccagtcatattaattactagtcaattagttgatttttatttttgacatatacatgtgaatgaaagaccccacctgtaggtttggcaagctagcttaagtaacgccattttgcaaggcatggaaaaatacataactgagaatagaaaagttcagatcaaggtcaggaacagatggaacagctgaatatgggccaaacaggatatctgtggtaagcagttcctgccccggctcagggccaagaacagatggaacagctgaatatgggccaaacaggatatctgtggtaagcagttcctgccccggctcagggccaagaacagatggtccccagatgcggtccagccctcagcagtttctagagaaccatcagatgtttccagggtgccccaaggacctgaaatgaccctgtgccttatttgaactaaccaatcagttcgcttctcgcttctgttcgcgcgcttatgctccccgagctcaataaaagagcccacaacccctcactcggggcgccagtcctccgattgactgagtcgcccgggtacccgtgtatccaataaaccctcttgcagttgcatccgacttgtggtctcgctgttccttgggagggtctcctctgagtgattgactacccgtcagcgggggtctttcatttgggggctcgtccgggatcgggagacccctgcccagggaccaccgacccaccaccgggaggtaagctggccagcaacttatctgtgtctgtccgattgtctagtgtctatgactgattttatgcgcctgcgtcggtactagttagctaactagctctgtatctggcggacccgtggtggaactgacgagttcggaacacccggccgcaaccctgggagacgtcccagggacttcgggggccgtttttgtggcccgacctgagtcctaaaatcccgatcgtttaggactctttggtgcaccccccttagaggagggatatgtggttctggtaggagacgagaacctaaaacagttcccgcctccgtctgaatttttgctttcggtttgggaccgaagccgcgccgcgcgtcttgtctgctgcagcatcgttctgtgttgtctctgtctgactgtgtttctgtatttgtctgaaaatatgggcccgggctagcctgttaccactcccttaagtttgaccttaggtcactggaaagatgtcgagcggatcgctcacaaccagtcggtagatgtcaagaagagacgttgggttaccttctgctctgcagaatggccaacctttaacgtcggatggccgcgagacggcacctttaaccgagacctcatcacccaggttaagatcaaggtcttttcacctggcccgcatggacacccagaccaggtggggtacatcgtgacctgggaagccttggcttttgacccccctccctgggtcaagccctttgtacaccctaagcctccgcctcctcttcctccatccgccccgtctctcccccttgaacctcctcgttcgaccccgcctcgatcctccctttatccagccctcactccttctctaggcgcccccatatggccatatgagatcttatatggggcacccccgccccttgtaaacttccctgaccctgacatgacaagagttactaacagcccctctctccaagctcacttacaggctctctacttagtccagcacgaagtctggagacctctggcggcagcctaccaagaacaactggaccgaccggtggtacctcacccttaccgagtcggcgacacagtgtgggtccgccgacaccagactaagaacctagaacctcgctggaaaggaccttacacagtcctgctgaccacccccaccgccctcaaagtagacggcatcgcagcttggatacacgccgcccacgtgaaggctgccgaccccgggggtggaccatcctctagactgccatggaagcccctgcccagctgctgttcctgctgctgctgtggctgcccgacaccaccggcgagatcgtgctgacacagagccccgccaccctgtctctgagccctggcgagagagccaccctgagctgtagcgccagcagcagcatcaactacatctactggctgcagcagaagcccggccaggcccccagaatcctgatctacctgaccagcaacctggccagcggcgtgcccgccagattttctggcagcggcagcggcaccgacttcaccctgaccatcagcagcctggaacccgaggacttcgccgtgtactactgcctgcagtggtccagcaaccccctgaccttcggcggaggcaccaaggtggaaatcaagcggggtggtggtggttctggtggtggtggttctgaggtgcagctggtggaaagcggcggaggcctggtcaagcctggcggcagcctgagactgagctgtgccgccagcggcttcaccttcagcagctacgacatgagctgggtccgacaggctccaggcaagggactggaatgggtgtccaccatcagcagcggcggcagctacacctactacctggacagcatcaagggccggttcaccatcagccgggacaacgccaagaacagcctgtacctgcagatgaacagcctgcgggccgaggacaccgccgtctactactgtgcccggcagggcctcgactactggggcagaggcaccctggtcaccgtgtccagcggggatcccaaagaggcctgccccaccggcctgtacacccacagcggagagtgctgcaaggcctgcaacctgggagagggcgtggcccagccttgcggcgccaatcagaccgtgtgcgagccctgcctggacagcgtgaccttcagcgacgtggtgtccgccaccgagccctgcaagccttgcaccgagtgtgtgggcctgcagagcatgagcgccccctgcgtggaagccgacgacgccgtgtgtagatgcgcctacggctactaccaggacgagacaaccggcagatgcgaggcctgtagagtgtgcgaggccggcagcggcctggtgttcagttgtcaggacaagcagaacaccgtgtgtgaagagtgccccgacggcacctacagcgacgaggccgcccgggccgccgacgccgagtgcgaggaacccaaattttgggtgctggtggtggttggtggagtcctggcttgctatagcttgctagtaacagtggcctttattattttctgggtgaggagtaagaggagcaggctcctgcacagtgactacatgaacatgactccccgccgccccgggcccacccgcaagcattaccagccctatgccccaccacgcgacttcgcagcctatcgctccagagtgaagttcagcaggagcgcagacgcccccgcgtaccagcagggccagaaccagctctataacgagctcaatctaggacgaagagaggagtacgatgttttggacaagagacgtggccgggaccctgagatggggggaaagccgagaaggaagaaccctcaggaaggcctgtacaatgaactgcagaaagataagatggcggaggcctacagtgagattgggatgaaaggcgagcgccggaggggcaaggggcacgatggcctttaccagggtctcagtacagccaccaaggacacctacgacgcccttcacatgcaggccctgcctcctcgctaagcatgcaacctcgatccggattagtccaatttgttaaagacaggatatcagtggtccaggctctagttttgactcaacaatatcaccagctgaagcctatagagtacgagccatagataaaataaaagattttatttagtctccagaaaaaggggggaatgaaagaccccacctgtaggtttggcaagctagcttaagtaacgccattttgcaaggcatggaaaaatacataactgagaatagagaagttcagatcaaggtcaggaacagatggaacagctgaatatgggccaaacaggatatctgtggtaagcagttcctgccccggctcagggccaagaacagatggaacagctgaatatgggccaaacaggatatctgtggtaagcagttcctgccccggctcagggccaagaacagatggtccccagatgcggtccagccctcagcagtttctagagaaccatcagatgtttccagggtgccccaaggacctgaaatgaccctgtgccttatttgaactaaccaatcagttcgcttctcgcttctgttcgcgcgcttctgctccccgagctcaataaaagagcccacaacccctcactcggggcgccagtcctccgattgactgagtcgcccgggtacccgtgtatccaataaaccctcttgcagttgcatccgacttgtggtctcgctgttccttgggagggtctcctctgagtgattgactacccgtcagcgggggtctttcacacatgcagcatgtatcaaaattaatttggttttttttcttaagtatttacattaaatggccatagtacttaaagttacattggcttccttgaaataaacatggagtattcagaatgtgtcataaatatttctaattttaagatagtatctccattggctttctactttttcttttatttttttttgtcctctgtcttccatttgttgttgttgttgtttgtttgtttgtttgttggttggttggttaatttttttttaaagatcctacactatagttcaagctagactattagctactctgtaacccagggtgaccttgaagtcatgggtagcctgctgttttagccttcccacatctaagattacaggtatgagctatcatttttggtatattgattgattgattgattgatgtgtgtgtgtgtgattgtgtttgtgtgtgtgactgtgaaaatgtgtgtatgggtgtgtgtgaatgtgtgtatgtatgtgtgtgtgtgagtgtgtgtgtgtgtgtgtgcatgtgtgtgtgtgtgactgtgtctatgtgtatgactgtgtgtgtgtgtgtgtgtgtgtgtgtgtgtgtgtgtgtgtgtgtgttgtgaaaaaatattctatggtagtgagagccaacgctccggctcaggtgtcaggttggtttttgagacagagtctttcacttagcttggaattcactggccgtcgttttacaacgtcgtgactgggaaaaccctggcgttacccaacttaatcgccttgcagcacatccccctttcgccagctggcgtaatagcgaagaggcccgcaccgatcgcccttcccaacagttgcgcagcctgaatggcgaatggcgcctgatgcggtattttctccttacgcatctgtgcggtatttcacaccgcatatggtgcactctcagtacaatctgctctgatgccgcatagttaagccagccccgacacccgccaacacccgctgacgcgccctgacgggcttgtctgctcccggcatccgcttacagacaagctgtgaccgtctccgggagctgcatgtgtcagaggttttcaccgtcatcaccgaaacgcgcgatgacgaaagggcctcgtgatacgcctatttttataggttaatgtcatgataataatggtttcttagacgtcaggtggcacttttcggggaaatgtgcgcggaacccctatttgtttatttttctaaatacattcaaatatgtatccgctcatgagacaataaccctgataaatgcttcaataatattgaaaaaggaagagtatgagtattcaacatttccgtgtcgcccttattcccttttttgcggcattttgccttcctgtttttgctcacccagaaacgctggtgaaagtaaaagatgctgaagatcagttgggtgcacgagtgggttacatcgaactggatctcaacagcggtaagatccttgagagttttcgccccgaagaacgttttccaatgatgagcacttttaaagttctgctatgtggcgcggtattatcccgtattgacgccgggcaagagcaactcggtcgccgcatacactattctcagaatgacttggttgagtactcaccagtcacagaaaagcatcttacggatggcatgacagtaagagaattatgcagtgctgccataaccatgagtgataacactgcggccaacttacttctgacaacgatcggaggaccgaaggagctaaccgcttttttgcacaacatgggggatcatgtaactcgccttgatcgttgggaaccggagctgaatgaagccataccaaacgacgagcgtgacaccacgatgcctgtagcaatggcaacaacgttgcgcaaactattaactggcgaactacttactctagcttcccggcaacaattaatagactggatggaggcggataaagttgcaggaccacttctgcgctcggcccttccggctggctggtttattgctgataaatctggagccggtgagcgtgggtctcgcggtatcattgcagcactggggccagatggtaagccctcccgtatcgtagttatctacacgacggggagtcaggcaactatggatgaacgaaatagacagatcgctgagataggtgcctcactgattaagcattggtaactgtcagaccaagtttactcatatatactttagattgatttaaaacttcatttttaatttaaaaggatctaggtgaagatcctttttgataatctcatgaccaaaatcccttaacgtgagttttcgttccactgagcgtcagaccccgtagaaaagatcaaaggatcttcttgagatcctttttttctgcgcgtaatctgctgcttgcaaacaaaaaaaccaccgctaccagcggtggtttgtttgccggatcaagagctaccaactctttttccgaaggtaactggcttcagcagagcgcagataccaaatactgtccttctagtgtagccgtagttaggccaccacttcaagaactctgtagcaccgcctacatacctcgctctgctaatcctgttaccagtggctgctgccagtggcgataagtcgtgtcttaccgggttggactcaagacgatagttaccggataaggcgcagcggtcgggctgaacggggggttcgtgcacacagcccagcttggagcgaacgacctacaccgaactgagatacctacagcgtgagcattgagaaagcgccacgcttcccgaagggagaaaggcggacaggtatccggtaagcggcagggtcggaacaggagagcgcacgagggagcttccagggggaaacgcctggtatctttatagtcctgtcgggtttcgccacctctgacttgagcgtcgatttttgtgatgctcgtcaggggggcggagcctatggaaaaacgccagcaacgcggcctttttacggttcctggccttttgctggccttttgctcacatgttctttcctgcgttatcccctgattctgtggataaccgtattaccgcctttgagtgagctgataccgctcgccgcagccgaacgaccgagcgcagcgagtcagtgagcgaggaagcggaagagcgcccaatacgcaaaccgcctctccccgcgcgttggccgattcattaatgcagctggcacgacaggtttcccgactggaaagcgggcagtgagcgcaacgcaattaatgtgagttagctcactcattaggcaccccaggctttacactttatgcttccggctcgtatgttgtgtggaattgtgagcggataacaatttcacacaggaaacagctatgaccatgattacgcc